European Patent Application EP 4 219 551 A1, published August 2, 2023. Title: ANTIBODY BINDING TO HUMAN IL-33, PREPARATION METHOD THEREOF, AND USE THEREOF. Applicant: Sunshine Guojian Pharmaceutical (Shanghai) Co., Ltd. The sequence listing filed with the application follows.

SEQUENCE LISTING (71 sequences)

SEQ ID NO: 1 - DNA, 363 bp, Mus musculus
caggtacagctgaaggagtcaggacctggcctggtggcgccctcacagagcctgtccatcacttgcactgtctctgggttttcattaaccaactatggtgtacactgggttcgcctgcctccaggaaagggtctggagtggctgggagtgatacgagctggtggaagttcagattataattcggctctcatgtccagactgaacatcaggaaagacaattccaagagccaagttttcttagaaatgaacagtcttcaaactgctgacacagccatgtactactgtgccagagaccattatttcagtaatagttacgggggttctccttactggggccaagggactctggtcactgtctctgca

SEQ ID NO: 2 - protein, 121 aa, Mus musculus
QVQLKESGPGLVAPSQSLSITCTVSGFSLTNYGVHWVRLPPGKGLEWLGVIRAGGSSDYNSALMSRLNIRKDNSKSQVFLEMNSLQTADTAMYYCARDHYFSNSYGGSPYWGQGTLVTVSA

SEQ ID NO: 3 - DNA, 363 bp, Mus musculus
caggttcacctgaaggagtcagggcctggcctggtggcgccctcacagagcctgtccatcacttgcaatgtctctggattttcattatccaaatatggtgtacactggatccgccagactccaggaaggggtctggactggctgggagtgttacgggctggtggaaccataagttataattcggctctcatgtccagactgagtatcagcgaagacatttccaaaagccaagttttcttaaaaatgaatgatttacaaactgatgactcagccatctacttctgtgccagagaccattactactatagttccttcgggggttttgcttcctggggtcaggggactctggtcactgtctctgca

SEQ ID NO: 4 - protein, 121 aa, Mus musculus
QVHLKESGPGLVAPSQSLSITCNVSGFSLSKYGVHWIRQTPGRGLDWLGVLRAGGTISYNSALMSRLSISEDISKSQVFLKMNDLQTDDSAIYFCARDHYYYSSFGGFASWGQGTLVTVSA

SEQ ID NO: 5 - DNA, 321 bp, Mus musculus
gacattcagatgacccagtctcctgcctcccagtctgcatctctgggagaaagtgtcaccatcacatgcctggcaagtcagaccattgctacatggttagcatggtatcagcagaaaccagggaaatctcctcagctcctgatttatgctgcaaccaggttggcagatggggtcccatcaaggttcagtggtagtggatctggcacagaattttctttcaagatcagtagcctacaggctgaagattttgtgatttattactgtcaacaactttacaatactccgtacacgttcggaggggggaccaagctggagataaaa

SEQ ID NO: 6 - protein, 107 aa, Mus musculus
DIQMTQSPASQSASLGESVTITCLASQTIATWLAWYQQKPGKSPQLLIYAATRLADGVPSRFSGSGSGTEFSFKISSLQAEDFVIYYCQQLYNTPYTFGGGTKLEIK

SEQ ID NO: 7 - DNA, 363 bp, Mus musculus
caggtgcaactgaaggagtcaggacctggtctggtggcgccctcacacagcctgtccatcacctgcaatgtctctgggttttcattatccaagtatggtgtacactggattcgtcagattccaggaaggggtctggactggctgggagtgttacgggctggtggaagtacaggttataattcggctctcatgtccaggctgagtatcagcaaagacagttccaaaagccaagttttcttaaagatgaacgatctacggactgatgacacagccgtttacttctgtgtcagagaccattactactacagttcttacgggggttttgtttactggggccaggggactctggtcactgtctctgca

SEQ ID NO: 8 - protein, 121 aa, Mus musculus
QVQLKESGPGLVAPSHSLSITCNVSGFSLSKYGVHWIRQIPGRGLDWLGVLRAGGSTGYNSALMSRLSISKDSSKSQVFLKMNDLRTDDTAVYFCVRDHYYYSSYGGFVYWGQGTLVTVSA

SEQ ID NO: 9 - DNA, 318 bp, Mus musculus
gacattcagatgacccagtctcctgcctcccagtctgcatctctgggagaaagtgtcaccatcacatgcctggcaagtcagaccataggtgcatggttagcatggtatcggcagcaaccaggaaaatctcctcagctcctgatttatgctgcaaccaggttggcagatggggtcccatcaaggttcagtggtagtggttctgggacagaattttctttcaagatcaacaacctacaggctgaagattttgtaagttattactgtcaacaacttgacagtagtccgtacacgttcggaggggggaccaggctggaaatg

SEQ ID NO: 10 - protein, 106 aa, Mus musculus
DIQMTQSPASQSASLGESVTITCLASQTIGAWLAWYRQQPGKSPQLLIYAATRLADGVPSRFSGSGSGTEFSFKINNLQAEDFVSYYCQQLDSSPYTFGGGTRLEM

SEQ ID NO: 11 - DNA, 318 bp, Mus musculus
gacattcagatgacccagtctcctgcctcccagtctgcatctctgggagaaagtgtcaccatcacatgcctggcaagtcagaccattggtgcatggttagcatggtatcggcagcaaccaggaaaatctcctcagctcctgatttatgctgcaaccaggttggcagatggggtcccatcaaggttcagtggtagtggatctggcacaaaattttctttcaagatcaacaacctacaggctgaagattttgtgatttattactgtcaacaacttaacagtactccgtacacgttcggaggggggaccaggctggaaatg

SEQ ID NO: 12 - protein, 106 aa, Mus musculus
DIQMTQSPASQSASLGESVTITCLASQTIGAWLAWYRQQPGKSPQLLIYAATRLADGVPSRFSGSGSGTKFSFKINNLQAEDFVIYYCQQLNSTPYTFGGGTRLEM

SEQ ID NO: 13 - protein, 327 aa, Human
ASTKGPSVFPLAPCSRSTSESTAALGCLVKDYFPEPVTVSWNSGALTSGVHTFPAVLQSSGLYSLSSVVTVPSSSLGTKTYTCNVDHKPSNTKVDKRVESKYGPPCPPCPAPEFLGGPSVFLFPPKPKDTLMISRTPEVTCVVVDVSQEDPEVQFNWYVDGVEVHNAKTKPREEQFNSTYRVVSVLTVLHQDWLNGKEYKCKVSNKGLPSSIEKTISKAKGQPREPQVYTLPPSQEEMTKNQVSLTCLVKGFYPSDIAVEWESNGQPENNYKTTPPVLDSDGSFFLYSRLTVDKSRWQEGNVFSCSVMHEALHNHYTQKSLSLSLGK

SEQ ID NO: 14 - protein, 107 aa, Human [sequence omitted]

SEQ ID NO: 15 - protein, 5 aa, Mus musculus
NYGVH

SEQ ID NO: 16 - protein, 16 aa, Mus musculus
VIRAGGSSDYNSALMS

SEQ ID NO: 17 - protein, 13 aa, Mus musculus
DHYFSNSYGGSPY

SEQ ID NO: 18 - protein, 5 aa, Mus musculus
KYGVH

SEQ ID NO: 19 - protein, 16 aa, Mus musculus
VLRAGGTISYNSALMS

SEQ ID NO: 20 - protein, 13 aa, Mus musculus
DHYYYSSFGGFAS

SEQ ID NO: 21 - protein, 11 aa, Mus musculus
LASQTIATWLA

SEQ ID NO: 22 - protein, 7 aa, Mus musculus
AATRLAD

SEQ ID NO: 23 - protein, 9 aa, Mus musculus
QQLYNTPYT

SEQ ID NO: 24 - protein, 16 aa, Mus musculus
VLRAGGSTGYNSALMS

SEQ ID NO: 25 - protein, 13 aa, Mus musculus
DHYYYSSYGGFVY

SEQ ID NO: 26 - protein, 11 aa, Mus musculus
LASQTIGAWLA

SEQ ID NO: 27 - protein, 9 aa, Mus musculus
QQLDSSPYT

SEQ ID NO: 28 - protein, 9 aa, Mus musculus
QQLNSTPYT

SEQ ID NO: 29 - protein, 121 aa, Composite
QVQLQESGPGLVKPSETLSLTCTVSGFSLTNYGVHWIRQPPGKGLEWIGVIRAGGSSDYNSALMSRVTISVDTSKNQFSLKLSSVTAADTAVYYCARDHYFSNSYGGSPYWGQGTLVTVSS

SEQ ID NO: 30 - protein, 121 aa, Composite
QVQLQESGPGLVKPSETLSLTCTVSGFSLTNYGVHWIRLPPGKGLEWIGVIRAGGSSDYNSALMSRVTISKDNSKSQVSLKLSSVTAADTAVYYCARDHYFSNSYGGSPYWGQGTLVTVSS

SEQ ID NO: 31 - protein, 121 aa, Composite
QVQLQESGPGLVKPSETLSLTCTVSGFSLTNYGVHWVRLPPGKGLEWLGVIRAGGSSDYNSALMSRLTISKDNSKSQVSLKLSSVTAADTAVYYCARDHYFSNSYGGSPYWGQGTLVTVSS

SEQ ID NO: 32 - protein, 107 aa, Composite
DIQMTQSPSSLSASVGDRVTITCLASQTIATWLAWYQQKPGKSPKLLIYAATRLADGVPSRFSGSGSGTDFTLTISSLQPEDFATYYCQQLYNTPYTFGQGTKVEIK

SEQ ID NO: 33 - protein, 121 aa, Composite
QVQLQESGPGLVKPSETLSLTCTVSGFSLSKYGVHWIRQPPGKGLEWIGVLRAGGTISYNSALMSRVTISVDTSKNQFSLKLSSVTAADTAVYYCARDHYYYSSFGGFASWGQGTLVTVSS

SEQ ID NO: 34 - protein, 121 aa, Composite
QVQLQESGPGLVKPSETLSLTCTVSGFSLSKYGVHWIRQPPGKGLEWIGVLRAGGTISYNSALMSRVTISEDISKSQVSLKLSSVTAADTAVYYCARDHYYYSSFGGFASWGQGTLVTVSS

SEQ ID NO: 35 - protein, 121 aa, Composite
QVQLQESGPGLVKPSETLSLTCTVSGFSLSKYGVHWIRQPPGKGLEWLGVLRAGGTISYNSALMSRLTISEDISKSQVSLKLSSVTAADTAVYYCARDHYYYSSFGGFASWGQGTLVTVSS

SEQ ID NO: 36 - protein, 107 aa, Composite
DIQMTQSPSSVSASVGDRVTITCLASQTIGAWLAWYQQKPGKSPKLLIYAATRLADGVPSRFSGSGSGTDFTLTISSLQPEDFATYYCQQLNSTPYTFGQGTKVEIK

SEQ ID NO: 37 - protein, 121 aa, Composite
QVQLQESGPGLVKPSETLSLTCTVSGFSLSKYGVHWIRQPPGKGLEWIGVLRAGGSTGYNSALMSRVTISVDTSKNQFSLKLSSVTAADTAVYYCARDHYYYSSYGGFVYWGQGTLVTVSS

SEQ ID NO: 38 - protein, 121 aa, Composite
QVQLQESGPGLVKPSETLSLTCTVSGFSLSKYGVHWIRQPPGKGLEWIGVLRAGGSTGYNSALMSRVTISKDTSKSQVSLKLSSVTAADTAVYYCARDHYYYSSYGGFVYWGQGTLVTVSS

SEQ ID NO: 39 - protein, 121 aa, Composite
QVQLQESGPGLVKPSETLSLTCTVSGFSLSKYGVHWIRQPPGKGLEWLGVLRAGGSTGYNSALMSRLTISKDSSKSQVSLKLSSVTAADTAVYYCVRDHYYYSSYGGFVYWGQGTLVTVSS

SEQ ID NO: 40 - protein, 107 aa, Composite
DIQMTQSPSSVSASVGDRVTITCLASQTIGAWLAWYQQKPGKSPKLLIYAATRLADGVPSRFSGSGSGTDFTLTISSLQPEDFATYYCQQLDSSPYTFGQGTKVEIK

SEQ ID NO: 41 - DNA, 363 bp, Composite
caggtgcagctgcaggagtctggaccaggcctggtgaagccttctgagaccctgagcctgacctgtaccgtgtccggctttagcctgacaaattatggcgtgcattggattagacagccacctggcaagggcctggagtggattggcgtgattagagctggaggttcctctgattataattctgctctgatgtctagggtgaccattagtgtggatacatctaagaatcagttttctctgaagctgagttctgtgactgccgctgatacagctgtgtattattgtgctagggaccattatttttctaatagctacggcggcagtccttactggggccagggcacactggtgaccgtgtctagc

SEQ ID NO: 42 - DNA, 363 bp, Composite
caggtgcagctgcaggagagcggccctggactggtgaagccatctgagactctgagcctgacctgtacagtgagcggattttctctgactaattacggagtgcattggattagactgcctccaggaaagggcctggaatggatcggtgtgattagagccggaggctcctctgattataattccgctttgatgtctagagtgaccatctctaaagataactctaagagtcaggtgtctctgaagctgagtagcgtgacagcagctgataccgctgtgtattactgcgccagggatcattacttttcaaactcttatggaggatctccttactggggccagggcaccctggtgacagtgagctct

SEQ ID NO: 43 - DNA, 363 bp, Composite
caggtgcagctgcaggagtctggccccggcctggtgaagccctccgagaccctgagcctgacttgcactgtgagtggctttagtctgactaattatggcgtgcattgggtgaggctgcctccaggcaagggactggagtggctgggagtgattagagctggtggatctagtgattataactccgctctgatgtccagactgaccatctctaaggacaactccaagagccaggtgtccctgaagctgtctagtgtgaccgccgccgacaccgccgtgtactactgcgccagggaccactacttttctaactcttacgggggctccccctactggggccagggcaccttggtgacagtgtctagc

SEQ ID NO: 44 - DNA, 321 bp, Composite
gatattcagatgacacagtctccttcttctctgtctgcttctgtgggagatagagtgaccattacctgcctggcttctcagaccattgccacatggctggcttggtatcagcagaagcctggaaagagccctaagctgctgatctatgctgctacaagactggctgatggcgtgccatctagattctccggatctggatccggaacagacttcaccctgacaatctcttctctgcagcctgaggatttcgctacctactattgccagcagctgtataatactccttatacatttggccagggcaccaaggtcgaaatcaag

SEQ ID NO: 45 - DNA, 363 bp, Composite
caggtgcagctgcaggaatctggacctggactggtgaagccatccgagacactgtctctgacatgtacagtgtctggcttttctctgtctaagtatggagtgcattggatcagacagcctcctggcaagggcctggagtggattggagtgctgagagctggcggaacaattagttataattctgctctgatgtctagagtgaccatcagcgtggatacctctaagaaccagttttctctgaagctgagttctgtgacagcagccgacactgctgtgtactactgtgctcgcgaccactactactacagctctttcggcggcttcgcctcctgggggcagggcaccctggtgaccgtgtcctcc

SEQ ID NO: 46 - DNA, 363 bp, Composite
caggtgcagctgcaggagtccggccctggcctggtgaagccctccgagaccctgagcctgacctgcaccgtgtccggcttctccctgtccaagtacggcgtgcactggatcaggcagcctcccggcaagggcctggagtggattggcgttctgagagctggaggcactatttcttataatagcgcactgatgtctagagtgacaatcagtgaggatatctctaagtcccaggtgagcctgaagttaagttctgtgacagctgctgacaccgctgtgtattattgtgctagggatcattactactactcttccttcggcggctttgcctcttggggccagggcaccctggttaccgtgagtagt

SEQ ID NO: 47 - DNA, 363 bp, Composite
caggtgcagctgcaggagagcggccccggcctggtgaagccctccgagaccctgagcctgacctgcaccgtgtccggcttttccctgagcaagtacggcgtgcactggatccgccagccccccggcaagggcctggagtggctgggcgtgctgagggccggcggcaccatcagctacaactccgccctgatgtcccggctgaccatctctgaggacatctccaagtcccaggtgtccctgaagctgagctccgtgaccgccgccgacaccgccgtgtactactgcgcccgcgaccactactactacagcagcttcggcggctttgccagctggggacagggcaccctggtgaccgtgagcagc

SEQ ID NO: 48 - DNA, 321 bp, Composite
gacatccagatgacccagtccccctcctccgtgtcggccagcgtgggcgacagagtgaccatcacctgcctggcctcccagacgatcggcgcctggctggcctggtaccagcagaagcccggcaagtcccccaagctgctgatctacgccgccaccagactggccgacggcgtgccctccaggttcagcggctccggatctggtaccgattttaccctgacaatctctagcctgcagcctgaggattttgccacatactactgtcagcagctgaatagtactccatacacctttggccagggaaccaaggtggagatcaag

SEQ ID NO: 49 - DNA, 363 bp, Composite
caggtgcagctgcaggagtccggccccggcctggtgaagccatccgagaccctgagccttacctgcaccgtgtctggcttcagcctgtctaagtacggcgtgcattggatcaggcagccccccggcaagggcctggagtggatcggcgtgctgagagccggcggcagcacaggctacaactccgccctgatgagcagggtgaccatcagcgtggacaccagcaagaaccagtttagcctgaagctgagcagcgtgaccgccgccgacaccgccgtgtactactgcgctcgggaccactactactactccagctacggcggcttcgtgtactggggccagggcaccctggtgaccgtgtctagc

SEQ ID NO: 50 - DNA, 363 bp, Composite
caggtgcagctgcaggagtctggccctggactggtgaagccttctgagacactgagtctgacatgtacagtgagtggcttctctctgtcgaagtatggagtgcactggattaggcagccccctggaaagggcctggagtggatcggcgtgctgcgggccggcggctctacgggctacaactccgccctgatgagccgggtgaccatcagcaaggacacctccaagagccaggtgagcctgaagctgtctagcgtgaccgccgccgacaccgccgtgtactactgcgccagggaccactactactattccagctatggcggcttcgtgtactggggccagggcaccctggtgaccgtgtcctcc

SEQ ID NO: 51 - DNA, 363 bp, Composite
caggtgcagctgcaggagagcggcccaggcctggtgaagccatctgaaaccctgtctctgacctgtacagtgtccggcttttccctgtctaaatacggtgtgcactggatcagacagcctcctggtaaaggcctggagtggctgggagtgctgagggctggaggaagtaccggctataatagcgctctgatgtctagattgactatctctaaggatagctctaaatctcaggtgagcctgaaactgagctctgtcaccgctgccgataccgctgtttattattgtgtgagggatcattactactactcctcttacggaggatttgtgtattggggtcagggcacactggtgacagtctcctct

SEQ ID NO: 52 - DNA, 321 bp, Composite
gacatccagatgacacagtctcctagctctgtgagcgcttctgtgggagatagagtgacaatcacctgtctggcttctcagaccattggagcttggctggcttggtaccagcagaaaccaggcaagtctcctaagctgctgatctatgctgctactagactggctgatggcgtgccatctagattttctggcagcggatctggaaccgattttacactgacaatctcttctctgcagcctgaggatttcgctacatactattgtcagcagctggattcttctccttacacatttggccagggaacaaaggtggaaattaag

SEQ ID NO: 53 - protein, 166 aa, Composite
MSITGISPITEYLASLSTYNDQSITFALEDESYEIYVEDLKKDEKKDKVLLSYYESQHPSNESGDGVDGKMLMVTLSPTKDFWLHANNKEHSVELHKCEKPLPDQAFFVLHNMHSNCVSFECKTDPGVFIGVKDNHLALIKVDSSENLCTENILFKLSETHHHHHH

SEQ ID NO: 54 - protein, 560 aa, Composite
MGFWILAILTILMYSTAAKFSKQSWGLENEALIVRCPRQGKPSYTVDWYYSQTNKSIPTQERNRVFASGQLLKFLPAAVADSGIYTCIVRSPTFNRTGYANVTIYKKQSDCNVPDYLMYSTVSGSEKNSKIYCPTIDLYNWTAPLEWFKNCQALQGSRYRAHKSFLVIDNVMTEDAGDYTCKFIHNENGANYSVTATRSFTVKDEQGFSLFPVIGAPAQNEIKEVEIGKNANLTCSACFGKGTQFLAAVLWQLNGTKITDFGEPRIQQEEGQNQSFSNGLACLDMVLRIADVKEEDLLLQYDCLALNLHGLRRHTVRLSRKNPSKECFENLYFQGTHTCPPCPAPELLGGPSVFLFPPKPKDTLMISRTPEVTCVVVDVSHEDPEVKFNWYVDGVEVHNAKTKPREEQYNSTYRVVSVLTVLHQDWLNGKEYKCKVSNKALPAPIEKTISKAKGQPREPQVYTLPPSRDELTKNQVSLTCLVKGFYPSDIAVEWESNGQPENNYKTTPPVLDSDGSFFLYSKLTVDKSRWQQGNVFSCSVMHEALHNHYTQKSLSLSPGK

SEQ ID NO: 55 - protein, 160 aa, human
MSITGISPITEYLASLSTYNDQSITFALEDESYEIYVEDLKKDEKKDKVLLSYYESQHPSNESGDGVDGKMLMVTLSPTKDFWLHANNKEHSVELHKCEKPLPDQAFFVLHNMHSNCVSFECKTDPGVFIGVKDNHLALIKVDSSENLCTENILFKLSET

SEQ ID NO: 56 - protein, 20 aa, Artificial Sequence
  Pep1
VQKYTRALHDSSITGISPIT

SEQ ID NO: 57 - protein, 20 aa, Artificial Sequence
  Pep2
SSITGISPITEYLASLSTYN

SEQ ID NO: 58 - protein, 20 aa, Artificial Sequence
  Pep3
EYLASLSTYNDQSITFALED

SEQ ID NO: 59 - protein, 20 aa, Artificial Sequence
  Pep4
DQSITFALEDESYEIYVEDL

SEQ ID NO: 60 - protein, 20 aa, Artificial Sequence
  Pep5
ESYEIYVEDLKKDEKKDKVL

SEQ ID NO: 61 - protein, 20 aa, Artificial Sequence
  Pep6
KKDEKKDKVLLSYYESQHPS

SEQ ID NO: 62 - protein, 20 aa, Artificial Sequence
  Pep7
LSYYESQHPSNESGDGVDGK

SEQ ID NO: 63 - protein, 20 aa, Artificial Sequence
  Pep8
NESGDGVDGKMLMVTLSPTK

SEQ ID NO: 64 - protein, 20 aa, Artificial Sequence
  Pep9
MLMVTLSPTKDFWLHANNKE

SEQ ID NO: 65 - protein, 20 aa, Artificial Sequence
  Pep10
DFWLHANNKEHSVELHKCEK

SEQ ID NO: 66 - protein, 20 aa, Artificial Sequence
  Pep11
HSVELHKCEKPLPDQAFFVL

SEQ ID NO: 67 - protein, 20 aa, Artificial Sequence
  Pep12
PLPDQAFFVLHNMHSNCVSF

SEQ ID NO: 68 - protein, 20 aa, Artificial Sequence
  Pep13
HNMHSNCVSFECKTDPGVFI

SEQ ID NO: 69 - protein, 20 aa, Artificial Sequence
  Pep14
ECKTDPGVFIGVKDNHLALI

SEQ ID NO: 70 - protein, 20 aa, Artificial Sequence
  Pep15
GVKDNHLALIKVDSSENLCT

SEQ ID NO: 71 - protein, 20 aa, Artificial Sequence
  Pep16
KVDSSENLCTENILFKLSET